European Patent Specification EP 3 811 979 B1, published November 29, 2023. Title: 抗Her2抗体药物偶联物药物制剂. Applicant: 荣昌生物制药（烟台）有限公司. The sequence listing filed with the application follows.

SEQUENCE LISTING (6 sequences)

SEQ ID NO: 1 - protein, 5 aa, Mus musculus
DYYIH

SEQ ID NO: 2 - protein, 17 aa, Mus musculus
RVNPDHGDSYYNQKFKD

SEQ ID NO: 3 - protein, 9 aa, Mus musculus
ARNYLFDHW

SEQ ID NO: 4 - protein, 11 aa, Mus musculus
KASQDVGTAVA

SEQ ID NO: 5 - protein, 7 aa, Mus musculus
WASIRHT

SEQ ID NO: 6 - protein, 7 aa, Mus musculus
HQFATYT